European Patent Application EP 4 606 390 A1, published August 27, 2025. Title: 酶裂解连接子及包含其的配体-艾瑞布林偶联物. Applicant: 英诺湖医药(杭州)有限公司. The sequence listing filed with the application follows.

SEQUENCE LISTING (15 sequences)

SEQ ID NO: 1 - protein, 5 aa, synthetic construct
SYAVS

SEQ ID NO: 2 - protein, 17 aa, synthetic construct
SISGGGIYIYYPDSVKG

SEQ ID NO: 3 - protein, 9 aa, synthetic construct
HGGAGYFDY

SEQ ID NO: 4 - protein, 11 aa, synthetic construct
RGSESVHSYLA

SEQ ID NO: 5 - protein, 7 aa, synthetic construct
NAKTLQS

SEQ ID NO: 6 - protein, 10 aa, synthetic construct
QQHYGSPPWT

SEQ ID NO: 7 - protein, 118 aa, synthetic construct
EVQLVESGGGLVKPGGSLRLSCAASGFTFSSYAVSWVRQAPGKGLEWVASISGGGIYIYYPDSVKGRFTISRDNAKNSLYLQMNSLRAEDTAVYYCARHGGAGYFDYWGQGTLVTVSS

SEQ ID NO: 8 - protein, 108 aa, synthetic construct
DSQMTQSPSSLSASVGDRVTITCRGSESVHSYLAWYQQKPGKAPKLLVYNAKTLQSGVPSRFSGSGSGTDFTLTISSLQPEDFATYYCQQHYGSPPWTFGGGTKVEIK

SEQ ID NO: 9 - protein, 330 aa, synthetic construct [sequence omitted]

SEQ ID NO: 10 - protein, 330 aa, synthetic construct
ASTKGPSVFPLAPSSKSTSGGTAALGCLVKDYFPEPVTVSWNSGALTSGVHTFPAVLQSSGLYSLSSVVTVPSSSLGTQTYICNVNHKPSNTKVDKKVEPKSCDKTHTSPPSPAPELLGGPSVFLFPPKPKDTLMISRTPEVTCVVVDVSHEDPEVKFNWYVDGVEVHNAKTKPREEQYNSTYRVVSVLTVLHQDWLNGKEYKCKVSNKALPAPIEKTISKAKGQPREPQVCTLPPCRDELTKNQVSLTCLVKGFYPSDIAVEWESNGQPENNYKTTPPVLDSDGSFFLYSKLTVDKSRWQQGNVFSCSVMHEALHNHYTQKSLSLSPGK

SEQ ID NO: 11 - protein, 107 aa, synthetic construct [sequence omitted]

SEQ ID NO: 12 - protein, 450 aa, synthetic construct
EVQLVESGGGLVQPGGSLRLSCAASGFNIKDTYIHWVRQAPGKGLEWVARIYPTNGYTRYADSVKGRFTISADTSKNTAYLQMNSLRAEDTAVYYCSRWGGDGFYAMDYWGQGTLVTVSSASTKGPSVFPLAPSSKSTSGGTAALGCLVKDYFPEPVTVSWNSGALTSGVHTFPAVLQSSGLYSLSSVVTVPSSSLGTQTYICNVNHKPSNTKVDKKVEPKSCDKTHTCPPCPAPELLGGPSVFLFPPKPKDTLMISRTPEVTCVVVDVSHEDPEVKFNWYVDGVEVHNAKTKPREEQYNSTYRVVSVLTVLHQDWLNGKEYKCKVSNKALPAPIEKTISKAKGQPREPQVYTLPPSREEMTKNQVSLTCLVKGFYPSDIAVEWESNGQPENNYKTTPPVLDSDGSFFLYSKLTVDKSRWQQGNVFSCSVMHEALHNHYTQKSLSLSPGK

SEQ ID NO: 13 - protein, 214 aa, synthetic construct
DIQMTQSPSSLSASVGDRVTITCRASQDVNTAVAWYQQKPGKAPKLLIYSASFLYSGVPSRFSGSRSGTDFTLTISSLQPEDFATYYCQQHYTTPPTFGQGTKVEIKRTVAAPSVFIFPPSDEQLKSGTASVVCLLNNFYPREAKVQWKVDNALQSGNSQESVTEQDSKDSTYSLSSTLTLSKADYEKHKVYACEVTHQGLSSPVTKSFNRGEC

SEQ ID NO: 14 - protein, 444 aa, synthetic construct
QVQLVQSGAEVKKPGSSVKVSCKASGYIFTTYNVHWVRQAPGQGLEWIGSIYPDNGDTSYNQNFKGRATITADKSTSTAYMELSSLRSEDTAVYYCARGDFAYWGQGTLVTVSSASTKGPSVFPLAPSSKSTSGGTAALGCLVKDYFPEPVTVSWNSGALTSGVHTFPAVLQSSGLYSLSSVVTVPSSSLGTQTYICNVNHKPSNTKVDKRVEPKSCDKTHTCPPCPAPELLGGPSVFLFPPKPKDTLMISRTPEVTCVVVDVSHEDPEVKFNWYVDGVEVHNAKTKPREEQYNSTYRVVSVLTVLHQDWLNGKEYKCKVSNKALPAPIEKTISKAKGQPREPQVYTLPPSREEMTKNQVSLTCLVKGFYPSDIAVEWESNGQPENNYKTTPPVLDSDGSFFLYSKLTVDKSRWQQGNVFSCSVMHEALHNHYTQKSLSLSPGK

SEQ ID NO: 15 - protein, 214 aa, synthetic construct
DIQMTQSPSSLSASVGDRVTITCKASQGVSNDVAWYQQKPGKAPKLLIYSASYRYTGVPSRFSGSGSGTDFTFTISSLQPEDIATYYCQQHSTTPYTFGQGTKLEIKRTVAAPSVFIFPPSDEQLKSGTASVVCLLNNFYPREAKVQWKVDNALQSGNSQESVTEQDSKDSTYSLSSTLTLSKADYEKHKVYACEVTHQGLSSPVTKSFNRGEC